European Patent Application EP 4 768 579 A2, published July 1, 2026. Title: Clostridium botulinum Serotype A Neurotoxin (BoNT/A) Sequence Variants. Applicant: AbbVie Inc. The sequence listing filed with the application follows.

SEQUENCE LISTING (4 sequences)

SEQ ID NO: 1 - protein, 1296 aa, Clostridium botulinum
  source 1..1296: note = amino acid sequence of the 150 kDa BoNT/A molecule
MPFVNKQFNYKDPVNGVDIAYIKIPNAGQMQPVKAFKIHNKIWVIPERDTFTNPEEGDLNPPPEAKQVPVSYYDSTYLSTDNEKDNYLKGVTKLFERIYSTDLGRMLLTSIVRGIPFWGGSTIDTELKVIDTNCINVIQPDGSYRSEELNLVIIGPSADIIQFECKSFGHEVLNLTRNGYGSTQYIRFSPDFTFGFEESLEVDTNPLLGAGKFATDPAVTLAHELIHAGHRLYGIAINPNRVFKVNTNAYYEMSGLEVSFEELRTFGGHDAKFIDSLQENEFRLYYYNKFKDIASTLNKAKSIVGTTASLQYMKNVFKEKYLLSEDTSGKFSVDKLKFDKLYKMLTEIYTEDNFVKFFKVLNRKTYLNFDKAVFKINIVPKVNYTIYDGFNLRNTNLAANFNGQNTEINNMNFTKLKNFTGLFEFYKLLCVRGIITSKTKSLDKGYNKALNDLCIKVNNWDLFFSPSEDNFTNDLNKGEEITSDTNIEAAEENISLDLIQQYYLTFNFDNEPENISIENLSSDIIGQLELMPNIERFPNGKKYELDKYTMFHYLRAQEFEHGKSRIALTNSVNEALLNPSRVYTFFSSDYVKKVNKATEAAMFLGWVEQLVYDFTDETSEVSTTDKIADITIIIPYIGPALNIGNMLYKDDFVGALIFSGAVILLEFIPEIAIPVLGTFALVSYIANKVLTVQTIDNALSKRNEKWDEVYKYIVTNWLAKVNTQIDLIRKKMKEALENQAEATKAIINYQYNQYTEEEKNNINFNIDDLSSKLNESINKAMININKFLNQCSVSYLMNSMIPYGVKRLEDFDASLKDALLKYIYDNRGTLIGQVDRLKDKVNNTLSTDIPFQLSKYVDNQRLLSTFTEYIKNIINTSILNLRYESNHLIDLSRYASKINIGSKVNFDPIDKNQIQLFNLESSKIEVILKNAIVYNSMYENFSTSFWIRIPKYFNSISLNNEYTIINCMENNSGWKVSLNYGEIIWTLQDTQEIKQRVVFKYSQMINISDYINRWIFVTITNNRLNNSKIYINGRLIDQKPISNLGNIHASNNIMFKLDGCRDTHRYIWIKYFNLFDKELNEKEIKDLYDNQSNSGILKDFWGDYLQYDKPYYMLNLYDPNKYVDVNNVGIRGYMYLKGPRGSVMTTNIYLNSSLYRGTKFIIKKYASGNKDNIVRNNDRVYINVVVKNKEYRLATNASQAGVEKILSALEIPDVGNLSQVVVMKSKNDQGITNKCKMNLQDNNGNDIGFIGFHQFNNIAKLVASNWYNRQIERSSRTLGCSWEFIPVDDGWGERPL

SEQ ID NO: 2 - protein, 437 aa, Clostridium botulinum
  source 1..437: note = amino acid sequence of the light chain (LC) of full-length 150 kDa BoNT/A
PFVNKQFNYKDPVNGVDIAYIKIPNAGQMQPVKAFKIHNKIWVIPERDTFTNPEEGDLNPPPEAKQVPVSYYDSTYLSTDNEKDNYLKGVTKLFERIYSTDLGRMLLTSIVRGIPFWGGSTIDTELKVIDTNCINVIQPDGSYRSEELNLVIIGPSADIIQFECKSFGHEVLNLTRNGYGSTQYIRFSPDFTFGFEESLEVDTNPLLGAGKFATDPAVTLAHELIHAGHRLYGIAINPNRVFKVNTNAYYEMSGLEVSFEELRTFGGHDAKFIDSLQENEFRLYYYNKFKDIASTLNKAKSIVGTTASLQYMKNVFKEKYLLSEDTSGKFSVDKLKFDKLYKMLTEIYTEDNFVKFFKVLNRKTYLNFDKAVFKINIVPKVNYTIYDGFNLRNTNLAANFNGQNTEINNMNFTKLKNFTGLFEFYKLLCVRGIITSK

SEQ ID NO: 3 - protein, 848 aa, Clostridium botulinum
  source 1..848: note = amino acid sequence of the heavy chain (HC) of 150 kDa BoNT/A
ALNDLCIKVNNWDLFFSPSEDNFTNDLNKGEEITSDTNIEAAEENISLDLIQQYYLTFNFDNEPENISIENLSSDIIGQLELMPNIERFPNGKKYELDKYTMFHYLRAQEFEHGKSRIALTNSVNEALLNPSRVYTFFSSDYVKKVNKATEAAMFLGWVEQLVYDFTDETSEVSTTDKIADITIIIPYIGPALNIGNMLYKDDFVGALIFSGAVILLEFIPEIAIPVLGTFALVSYIANKVLTVQTIDNALSKRNEKWDEVYKYIVTNWLAKVNTQIDLIRKKMKEALENQAEATKAIINYQYNQYTEEEKNNINFNIDDLSSKLNESINKAMININKFLNQCSVSYLMNSMIPYGVKRLEDFDASLKDALLKYIYDNRGTLIGQVDRLKDKVNNTLSTDIPFQLSKYVDNQRLLSTFTEYIKNIINTSILNLRYESNHLIDLSRYASKINIGSKVNFDPIDKNQIQLFNLESSKIEVILKNAIVYNSMYENFSTSFWIRIPKYFNSISLNNEYTIINCMENNSGWKVSLNYGEIIWTLQDTQEIKQRVVFKYSQMINISDYINRWIFVTITNNRLNNSKIYINGRLIDQKPISNLGNIHASNNIMFKLDGCRDTHRYIWIKYFNLFDKELNEKEIKDLYDNQSNSGILKDFWGDYLQYDKPYYMLNLYDPNKYVDVNNVGIRGYMYLKGPRGSVMTTNIYLNSSLYRGTKFIIKKYASGNKDNIVRNNDRVYINVVVKNKEYRLATNASQAGVEKILSALEIPDVGNLSQVVVMKSKNDQGITNKCKMNLQDNNGNDIGFIGFHQFNNIAKLVASNWYNRQIERSSRTLGCSWEFIPVDDGWGERPL

SEQ ID NO: 4 - protein, 435 aa, Clostridium botulinum
  source 1..435: note = amino acid sequence of the light chain (LC) of the truncated 150 kDa BoNT/A with C-terminal (-SK) truncation
PFVNKQFNYKDPVNGVDIAYIKIPNAGQMQPVKAFKIHNKIWVIPERDTFTNPEEGDLNPPPEAKQVPVSYYDSTYLSTDNEKDNYLKGVTKLFERIYSTDLGRMLLTSIVRGIPFWGGSTIDTELKVIDTNCINVIQPDGSYRSEELNLVIIGPSADIIQFECKSFGHEVLNLTRNGYGSTQYIRFSPDFTFGFEESLEVDTNPLLGAGKFATDPAVTLAHELIHAGHRLYGIAINPNRVFKVNTNAYYEMSGLEVSFEELRTFGGHDAKFIDSLQENEFRLYYYNKFKDIASTLNKAKSIVGTTASLQYMKNVFKEKYLLSEDTSGKFSVDKLKFDKLYKMLTEIYTEDNFVKFFKVLNRKTYLNFDKAVFKINIVPKVNYTIYDGFNLRNTNLAANFNGQNTEINNMNFTKLKNFTGLFEFYKLLCVRGIIT